European Patent Application EP 4 737 567 A2, published May 6, 2026. Title: Vaccine composition against Streptococcus suis infection. Applicant: Ceva Santé animale. Application EP. The sequence listing filed with the application follows.

SEQUENCE LISTING (14 sequences)

SEQ ID NO: 1 - protein, 1141 aa, Streptococcus suis
MNIQERFSLRKSAVGLVSVSLLCAIYTSTVAADTVVTGVNEIIEESQVKDEVSIESEKNESLDGSNIEIVEEIADNIPSPVIAEGEVAVEMKVDRGTENVVSRNDTEVTTSEQNQIEVTETKEILNQTSYQTESGEQRQIIWAHGITPPAMEQSGGFVKEKYGDYLNYTAPFEAGKGYYDTNKSLNASFIDLNLCFAAVSSNMVHWWLEQNSSYVERYLKEKKGTVNVEENYAITDLRRYINSFQNQQNSRVFDMFKTYYGYRTNGFVSDALVDLFINGYKPKAQGGVNLEDSQLVPDSRGGFFYDVFKEKKLTNRIFSGSYERFGEDVRTVLESKGLLGLTYRTLGYATHIVTVWGAEYDNQGKIKAVYITDSDDQQEQIGLKRMGITRDASGNPRLNNHMKNNSAGALLDYVHTIRLGQDLWEEYFNPLAKAKETASQTLADTKKALDLSIQGQSELPESMRLIYLEKLNNLYNQGILSIQKAESSEMLSGALENGLNSLKSLDFPISEVGNALAPDLPVGDRSTVSDVDSLSSQETSSTNLEADTENAGIIADGTNQLHFPVEAQTTSSVEAEGDNVFEQEADTLPIIIENKDEFGSELSRNMQTSETDSLVVAVEEDVKNDEVAQVEELLESEKVENQSSELLSDTLIVESANDKEEDRVEAVVSEQPDSIPHQNVEISLVEPTNVETETVVTPINDAATPHGSPTYIDNSVTESVATPLEKDSIQAGETEIAEPTSSESTNVETETVVTPVNDVATPHGSPTYIDNSVTESVATPLEKDSIQAGETEIAEPTSSESTNVETETVVTPVNDVATPHGSPTYIDNSVTESVATPLEKDSIQAGETEIAEPTSSESTSVEAELVDNSEIHAATSSVTPCGSSAYADGSTTESVATPLEKDSIQTGNTEIAEPTSSKSTNVEAASVDNSEIHADASLTAVSSVNLDNPVIEPVAISLIGSKRDTNAEVEVSSLSKREVRKTNTDGLISVQSKVIKKELLESSLAEAGSPLLEATIAQSSNSNSTEIGMSYQNTVLLESNNTERQVSKAEIVMEHKETELVETVSSASEPVVLVENISQTSNNTIESGKNMGVQSQAGAKQILGVEQSSKVSTPTSRQIMGVGLLTLVLGSALGLLKKRRK

SEQ ID NO: 2 - protein, 1130 aa, synthetic construct
  REGION 1..1130: note = rIdeSsuis
MAHHHHHHVGTGSNDDDDKSPDPVVTGVNEIIEESQVKDEVSIESEKNESLDGSNIEIVEEIADNIPSPVIAEGEVAVEMKVDRGTENVVSRNDTEVTTSEQNQIEVTETKEILNQTSYQTESGEQRQIIWAHGITPPAMEQSGGFVKEKYGDYLNYTAPFEAGKGYYDTNKSLNASFIDLNLCFAAVSSNMVHWWLEQNSSYVERYLKEKKGTVNVEENYAITDLRRYINSFQNQQNSRVFDMFKTYYGYRTNGFVSDALVDLFINGYKPKAQGGVNLEDSQLVPDSRGGFFYDVFKEKKLTNRIFSGSYERFGEDVRTVLESKGLLGLTYRTLGYATHIVTVWGAEYDNQGKIKAVYITDSDDQQEQIGLKRMGITRDASGNPRLNNHMKNNSAGALLDYVHTIRLGQDLWEEYFNPLAKAKETASQTLADTKKALDLSIQGQSELPESMRLIYLEKLNNLYNQGILSIQKAESSEMLSGALENGLNSLKSLDFPISEVGNALAPDLPVGDRSTVSDVDSLSSQETSSTNLEADTENAGIIADGTNQLHFPVEAQTTSSVEAEGDNVFEQEADTLPIIIENKDEFGSELSRNMQTSETDSLVVAVEEDVKNDEVAQVEELLESEKVENQSSELLSDTLIVESANDKEEDRVEAVVSEQPDSIPHQNVEISLVEPTNVETETVVTPINDAATPHGSPTYIDNSVTESVATPLEKDSIQAGETEIAEPTSSESTNVETETVVTPVNDVATPHGSPTYIDNSVTESVATPLEKDSIQAGETEIAEPTSSESTNVETETVVTPVNDVATPHGSPTYIDNSVTESVATPLEKDSIQAGETEIAEPTSSESTSVEAELVDNSEIHAATSSVTPCGSSAYADGSTTESVATPLEKDSIQTGNTEIAEPTSSKSTNVEAASVDNSEIHADASLTAVSSVNLDNPVIEPVAISLIGSKRDTNAEVEVSSLSKREVRKTNTDGLISVQSKVIKKELLESSLAEAGSPLLEATIAQSSNSNSTEIGMSYQNTVLLESNNTERQVSKAEIVMEHKETELVETVSSASEPVVLVENISQTSNNTIESGKNMGVQSQAGAKQILGVEQSSKVSTPTSRQIMGVGLLTLVLGSALGLLKKRRK

SEQ ID NO: 3 - DNA, 3426 bp, Streptococcus suis
  source 1..3426: mol_type = other DNA
atgaacattcaagaacgattttctttgagaaaatccgcggttggcttggtctcagtctctttgctatgtgctatttatacatccactgttgctgccgatacagttgttacaggagtgaatgaaataattgaagaatcacaagtcaaggatgaggtatctattgaatcagaaaaaaatgaatccctagatggttctaatattgaaattgtagaggaaatagcagacaacatcccatcacctgttatcgctgaaggggaagtagcggtagagatgaaagttgacagagggaccgagaatgtagtttctagaaatgatacagaagttacgacgagcgagcaaaatcagatagaggttactgagacaaaagaaattttgaatcagaccagttatcaaacggagagtggcgagcaacgacaaattatatgggcccatggaattactcctcctgcaatggaacaaagcggtggttttgtaaaggaaaagtatggagactatttaaactatacagcgccatttgaggctggaaaaggctactatgataccaataagagtctgaatgcttcatttattgaccttaatctttgttttgcagctgtgtcttcaaacatggtacattggtggttggaacagaatagttcctatgttgagcgatatctcaaagaaaaaaagggtacagtaaatgttgaagaaaactacgcaataacggacttacggcgctatattaattcattccaaaatcaacaaaatagtcgagtttttgatatgttcaaaacttactatggttatcgtacaaatggttttgtatcagatgccttggttgacttgtttattaacggatataaacctaaggcacagggcggtgtcaatctggaagatagccagttagtaccagatagtaggggtggctttttctacgacgttttcaaagagaaaaaactgacaaatcgaatttttagtggtagttatgagcggtttggtgaggatgttcgaactgttttggaaagcaaaggattactcggcttaacttatagaacattaggttatgcaacgcatattgtgacggtatggggtgctgagtacgacaatcaaggtaagattaaggctgtctatatcacagattctgatgatcaacaagaacaaattggtttgaagcgtatgggaatcactcgtgatgcttccggaaatccacgtttgaataatcatatgaaaaataattcagctggagcgcttttggattatgtccatacaatccgtctgggtcaagacttatgggaagaatatttcaatccgcttgcaaaagccaaagaaacagctagtcagacattagccgatacaaagaaggcgttggatttgtctattcaaggacaatctgaattgccagaatcaatgcgactgatttatcttgaaaaactaaataatctctataatcaaggaattctatctattcaaaaggcagaaagttctgagatgctaagtggtgcattggaaaatggtttaaatagtttaaagagtttagattttcctatttcagaagttggaaatgctttggcaccagatttaccagtaggtgatcgctcaacggtttcagatgttgattctctatcatctcaagaaacaagttccacaaatttggaagcagacacagagaatgcaggtattattgcagatggtaccaatcaattgcattttccagtggaggcccaaacgacatcttcagtagaggctgagggagataatgtttttgaacaagaggcagatacattaccaataattattgaaaacaaggatgaatttggttcagaactatcaagaaacatgcaaacgtcagaaacggattcgctagtagtagctgttgaagaagatgtgaaaaatgatgaggtagcccaagttgaagagcttcttgaatcagaaaaagttgaaaatcagagttcggaacttctgtcagacaccctaatcgtagagagtgcaaatgacaaagaagaagatagagtggaggcggttgtttctgaacaaccagactcaataccacatcaaaatgtagaaatctctcttgtagaaccaacgaatgtcgaaactgaaactgtggtcactcctattaatgatgcagctactcctcatggttccccgacgtatatagataattccgtaactgaatctgtagctactccacttgaaaaagactccattcaagccggggagacagagattgcagaaccaacctcgagcgaatcaacgaatgtcgaaactgaaactgtggtcactcctgttaatgatgtagctactcctcatggttccccgacgtatatagataattccgtaactgaatctgtagctactccacttgaaaaagactccattcaagccggagagacagaaattgcagaaccaacctcgagcgaatcaacgaatgtcgaaactgaaactgtggtcactcctgttaatgatgtagctactcctcatggttccccgacgtatatagataattccgtaactgaatctgtagctactccacttgaaaaagactccattcaagccggggagacagagattgcagaaccaacctcgagcgaatcaactagtgttgaagctgaacttgtcgacaattctgaaattcatgcagctacctcttcagttactccctgtggctcctcggcatatgcagatggttccacaactgaatctgtagccactccgcttgaaaaagactccattcagactggaaatacagaaattgcagaaccaacctcgagcaaatcaactaatgtagaagctgcatctgtcgacaattctgaaattcatgcagatgcctctctaactgctgtttcatcagttaatctggataatccagtgattgaaccagtagctatctcccttatcggttctaagagggacacgaatgcagaagtagaagtttcttcattatcgaaaagagaggttagaaaaacaaatactgacgggctaatctctgttcaatcaaaagttattaagaaagaattgctagaatcaagcttagcagaagcagggtctccattgctagaagccaccattgctcagtcttcaaactcaaatagtactgagataggtatgagctatcagaatactgtgttattagagtctaataatacagagcgtcaggtgtctaaagcagaaattgttatggaacacaaggagacagagttagttgaaacggtttcatctgcttctgagcctgtagtgctcgtagaaaatatctcacaaacctcaaataatactattgaatctggtaagaatatgggagttcaatctcaagcaggtgcaaaacaaattttaggcgtagaacaatcttcgaaagtaagtacacctacttcaagacagattatgggagtcggtctattgactcttgttcttggtagtgctttaggtttgttaaagaaaagacgtaagtaa

SEQ ID NO: 4 - DNA, 3393 bp, synthetic construct
  misc_feature 1..3393: note = Nucleotide sequence encoding rIdeSsuis
  source 1..3393: mol_type = other DNA
atggcacatcaccaccaccatcacgtgggtaccggttcgaatgatgacgacgacaagagtccggatccagttgttacaggagtgaatgaaataattgaagaatcacaagtcaaggatgaggtatctattgaatcagaaaaaaatgaatccctagatggttctaatattgaaattgtagaggaaatagcagacaacatcccatcacctgttatcgctgaaggggaagtagcggtagagatgaaagttgacagagggaccgagaatgtagtttctagaaatgatacagaagttacgacgagcgagcaaaatcagatagaggttactgagacaaaagaaattttgaatcagaccagttatcaaacggagagtggcgagcaacgacaaattatatgggcccatggaattactcctcctgcaatggaacaaagcggtggttttgtaaaggaaaagtatggagactatttaaactatacagcgccatttgaggctggaaaaggctactatgataccaataagagtctgaatgcttcatttattgaccttaatctttgttttgcagctgtgtcttcaaacatggtacattggtggttggaacagaatagttcctatgttgagcgatatctcaaagaaaaaaagggtacagtaaatgttgaagaaaactacgcaataacggacttacggcgctatattaattcattccaaaatcaacaaaatagtcgagtttttgatatgttcaaaacttactatggttatcgtacaaatggttttgtatcagatgccttggttgacttgtttattaacggatataaacctaaggcacagggcggtgtcaatctggaagatagccagttagtaccagatagtaggggtggctttttctacgacgttttcaaagagaaaaaactgacaaatcgaatttttagtggtagttatgagcggtttggtgaggatgttcgaactgttttggaaagcaaaggattactcggcttaacttatagaacattaggttatgcaacgcatattgtgacggtatggggtgctgagtacgacaatcaaggtaagattaaggctgtctatatcacagattctgatgatcaacaagaacaaattggtttgaagcgtatgggaatcactcgtgatgcttccggaaatccacgtttgaataatcatatgaaaaataattcagctggagcgcttttggattatgtccatacaatccgtctgggtcaagacttatgggaagaatatttcaatccgcttgcaaaagccaaagaaacagctagtcagacattagccgatacaaagaaggcgttggatttgtctattcaaggacaatctgaattgccagaatcaatgcgactgatttatcttgaaaaactaaataatctctataatcaaggaattctatctattcaaaaggcagaaagttctgagatgctaagtggtgcattggaaaatggtttaaatagtttaaagagtttagattttcctatttcagaagttggaaatgctttggcaccagatttaccagtaggtgatcgctcaacggtttcagatgttgattctctatcatctcaagaaacaagttccacaaatttggaagcagacacagagaatgcaggtattattgcagatggtaccaatcaattgcattttccagtggaggcccaaacgacatcttcagtagaggctgagggagataatgtttttgaacaagaggcagatacattaccaataattattgaaaacaaggatgaatttggttcagaactatcaagaaacatgcaaacgtcagaaacggattcgctagtagtagctgttgaagaagatgtgaaaaatgatgaggtagcccaagttgaagagcttcttgaatcagaaaaagttgaaaatcagagttcggaacttctgtcagacaccctaatcgtagagagtgcaaatgacaaagaagaagatagagtggaggcggttgtttctgaacaaccagactcaataccacatcaaaatgtagaaatctctcttgtagaaccaacgaatgtcgaaactgaaactgtggtcactcctattaatgatgcagctactcctcatggttccccgacgtatatagataattccgtaactgaatctgtagctactccacttgaaaaagactccattcaagccggggagacagagattgcagaaccaacctcgagcgaatcaacgaatgtcgaaactgaaactgtggtcactcctgttaatgatgtagctactcctcatggttccccgacgtatatagataattccgtaactgaatctgtagctactccacttgaaaaagactccattcaagccggagagacagaaattgcagaaccaacctcgagcgaatcaacgaatgtcgaaactgaaactgtggtcactcctgttaatgatgtagctactcctcatggttccccgacgtatatagataattccgtaactgaatctgtagctactccacttgaaaaagactccattcaagccggggagacagagattgcagaaccaacctcgagcgaatcaactagtgttgaagctgaacttgtcgacaattctgaaattcatgcagctacctcttcagttactccctgtggctcctcggcatatgcagatggttccacaactgaatctgtagccactccgcttgaaaaagactccattcagactggaaatacagaaattgcagaaccaacctcgagcaaatcaactaatgtagaagctgcatctgtcgacaattctgaaattcatgcagatgcctctctaactgctgtttcatcagttaatctggataatccagtgattgaaccagtagctatctcccttatcggttctaagagggacacgaatgcagaagtagaagtttcttcattatcgaaaagagaggttagaaaaacaaatactgacgggctaatctctgttcaatcaaaagttattaagaaagaattgctagaatcaagcttagcagaagcagggtctccattgctagaagccaccattgctcagtcttcaaactcaaatagtactgagataggtatgagctatcagaatactgtgttattagagtctaataatacagagcgtcaggtgtctaaagcagaaattgttatggaacacaaggagacagagttagttgaaacggtttcatctgcttctgagcctgtagtgctcgtagaaaatatctcacaaacctcaaataatactattgaatctggtaagaatatgggagttcaatctcaagcaggtgcaaaacaaattttaggcgtagaacaatcttcgaaagtaagtacacctacttcaagacagattatgggagtcggtctattgactcttgttcttggtagtgctttaggtttgttaaagaaaagacgtaagtaa

SEQ ID NO: 5 - protein, 335 aa, synthetic construct
  REGION 1..335: note = Partial sequence of Mac-1 domain
MKVDRGTENVVSRNDTEVTTSEQNQIEVTETKEILNQTSYQTESGEQRQIIWAHGITPPAMEQSGGFVKEKYGDYLNYTAPFEAGKGYYDTNKSLNASFIDLNLCFAAVSSNMVHWWLEQNSSYVERYLKEKKGTVNVEENYAITDLRRYINSFQNQQNSRVFDMFKTYYGYRTNGFVSDALVDLFINGYKPKAQGGVNLEDSQLVPDSRGGFFYDVFKEKKLTNRIFSGSYERFGEDVRTVLESKGLLGLTYRTLGYATHIVTVWGAEYDNQGKIKAVYITDSDDQQEQIGLKRMGITRDASGNPRLNNHMKNNSAGALLDYVHTIRLGQDLWE

SEQ ID NO: 6 - protein, 457 aa, synthetic construct
  REGION 1..457: note = rIdeSsuis_homologue
MAHHHHHHVGTGSNDDDDKSPDPVVTGVNEIIEESQVKDEVSIESEKNESLDGSNIEIVEEIADNIPSPVIAEGEVAVEMKVDRGTENVVSRNDTEVTTSEQNQIEVTETKEILNQTSYQTESGEQRQIIWAHGITPPAMEQSGGFVKEKYGDYLNYTAPFEAGKGYYDTNKSLNASFIDLNLCFAAVSSNMVHWWLEQNSSYVERYLKEKKGTVNVEENYAITDLRRYINSFQNQQNSRVFDMFKTYYGYRTNGFVSDALVDLFINGYKPKAQGGVNLEDSQLVPDSRGGFFYDVFKEKKLTNRIFSGSYERFGEDVRTVLESKGLLGLTYRTLGYATHIVTVWGAEYDNQGKIKAVYITDSDDQQEQIGLKRMGITRDASGNPRLNNHMKNNSAGALLDYVHTIRLGQDLWEEYFNPLAKACRSTSLRPHSSLVKKPLLRNLNASTWTRLLAQLN

SEQ ID NO: 7 - protein, 1016 aa, synthetic construct
  REGION 1..1016: note = rIdeSsuisB2
MAHHHHHHVGTGSNDDDDKSPDPVVTGVNEIIEESQVKDEVSIESEKNESLDGSNIEIVEEIADNIPSPVIAEGEVAVEMKVDRGTENVVSRNDTEVTTSEQNQIEVTETKEILNQTSYQTESGEQRQIIWAHGITPPAMEQSGGFVKEKYGDYLNYTAPFKAGKGYYDTNKSLNASFIDLNLCFAAVSSNMVHWWLEQNSSYVERYLKEKKGTVNVGENYAITDLRRYIDSFQDQQNSRVFDMFKTYYGYRTNGFVSDALVDLFINGYKPKVQGGVNLEDSQLVPDSRGGFFYDVFKEKKLTNRIFSGSYERFGEDVRTVLESKGLLGLTYRTLGYATHIVTVWGAEYDNQGKIRAVYITDSDDQQEQIGLKRMGITRDASGNPRLNNHVKNNSAGALLDYVHTIRLGQDLWEEYFNPFAKAKEIASQILADRKKALVLSIQGQSELPESMRLIYLEKLNNLYNQGILSIQKTESSEMLSGALENGLNSLKSLDFPISEVGNALAPDLSVGDRSTVSDVDSLSSQETSSTNLEADTENAGIIADGTNQLHFPVEAQTTSSVEAEGDNVFEQEADTLPIIIENKDEFGSELSGNMQTSETDSLVVAVEEDVKNDEVDQVEKLLESEKVENQSSELLSDTLIVEGANDKEEDRVEAVVSEQPDSIPHQNVEISPVEPMNVETESVVTPINDAATPHGFPMYIDNSVTESVATPLEKDSIQAGETEIAEPTSSESTSVEAELVDNSEIHSATSSVTPRGSSAYADSSTTESVATLLEKDSIQAGETEIAEPTSSKSTNVEAASVDNSEIHADTSLTAVSSVNLDNPVIEPVAIPLIGSKRDTNAEVEVSSLSKREVRKPNTEGLISVQSKVIKKELLESSLVEAGSPLLEATIAQSSNSNSTEIGMSYQNTVLLESNNTERQVSKAEIVIEHKETELVETVSSASEPVVLVENISQTSNNTIESGKNMGVQSQAGAKQILGIEQSSKVSTPTSRQIMGVGLLTLVLGSALGLLKKRRK

SEQ ID NO: 8 - DNA, 1374 bp, synthetic construct
  misc_feature 1..1374: note = Nucleotide sequence encoding rIdeSsuis_homologue
  source 1..1374: mol_type = other DNA
atggcacatcaccaccaccatcacgtgggtaccggttcgaatgatgacgacgacaagagtccggatccagttgttacaggagtgaatgaaataattgaagaatcacaagtcaaggatgaggtatctattgaatcagaaaaaaatgaatccctagatggttctaatattgaaattgtagaggaaatagcagacaacatcccatcacctgttatcgctgaaggggaagtagcggtagagatgaaagttgacagagggaccgagaatgtagtttctagaaatgatacagaagttacgacgagcgagcaaaatcagatagaggttactgagacaaaagaaattttgaatcagaccagttatcaaacggagagtggcgagcaacgacaaattatatgggcccatggaattactcctcctgcaatggaacaaagcggtggttttgtaaaggaaaagtatggagactatttaaactatacagcgccatttgaggctggaaaaggctactatgataccaataagagtctgaatgcttcatttattgaccttaatctttgttttgcagctgtgtcttcaaacatggtacattggtggttggaacagaatagttcctatgttgagcgatatctcaaagaaaaaaagggtacagtaaatgttgaagaaaactacgcaataacggacttacggcgctatattaattcattccaaaatcaacaaaatagtcgagtttttgatatgttcaaaacttactatggttatcgtacaaatggttttgtatcagatgccttggttgacttgtttattaacggatataaacctaaggcacagggcggtgtcaatctggaagatagccagttagtaccagatagtaggggtggctttttctacgacgttttcaaagagaaaaaactgacaaatcgaatttttagtggtagttatgagcggtttggtgaggatgttcgaactgttttggaaagcaaaggattactcggcttaacttatagaacattaggttatgcaacgcatattgtgacggtatggggtgctgagtacgacaatcaaggtaagattaaggctgtctatatcacagattctgatgatcaacaagaacaaattggtttgaagcgtatgggaatcactcgtgatgcttccggaaatccacgtttgaataatcatatgaaaaataattcagctggagcgcttttggattatgtccatacaatccgtctgggtcaagacttatgggaagaatatttcaatccgcttgcaaaagcctgcaggtcgacaagcttgcggccgcactcgagtctggtaaagaaaccgctgctgcgaaatttgaacgccagcacatggactcgtctactagcgcagcttaattaa

SEQ ID NO: 9 - DNA, 3051 bp, synthetic construct
  misc_feature 1..3051: note = Nucleotide sequence encoding rIdeSsuisB2
  source 1..3051: mol_type = other DNA
atggcacatcaccaccaccatcacgtgggtaccggttcgaatgatgacgacgacaagagtccggatccagttgttacaggagtgaatgaaataattgaagaatcacaagtcaaggatgaggtatctattgaatcagaaaaaaatgaatccctagatggttctaatattgaaattgtagaggaaatagcagacaacatcccatcacctgttatcgctgaaggggaagtagcggtagagatgaaagttgacagagggaccgagaatgtagtttctagaaatgatacagaagttacgacgagcgagcaaaatcagatagaggttactgagacaaaagaaattttgaatcagaccagttatcaaacggagagtggcgagcaacgacaaattatatgggcccatggaattactcctcctgcaatggaacaaagcggtggttttgtaaaggaaaagtatggagactatttaaactatacagcgccatttaaggcaggaaaaggctattatgataccaataaaagtctcaatgcttcatttattgaccttaacctatgttttgcagccgtgtcttccaacatggtacattggtggttggaacagaatagttcctatgttgagcgatatctcaaagaaaaaaagggtacagtaaatgttggggaaaactatgcaataacggacctacgtcgctatattgattcgttccaggatcagcaaaatagtcgagtctttgatatgttcaaaacttactacggttatcgtacaaatggttttgtgtcagatgccctagttgacttgtttattaatggatataaacctaaggtacagggtggtgtcaatctggaagatagccagttagtaccagatagtaggggtggctttttctacgacgttttcaaagagaaaaaactgacaaatcgtatttttagtggtagctatgagcgttttggtgaggatgttcgaactgttttggagagcaaaggattactcggtctaacttatagaacattaggctatgcaacgcatattgtgacggtatggggtgctgagtacgataatcaaggtaagattagggctgtctatatcactgattccgatgatcaacaagaacaaattggtttgaagcgtatgggaatcactcgtgatgcttctggaaatccgcgtttgaataatcatgtgaaaaataattcagctggggcgcttttggattatgtccatacaatccgtcttggtcaagacttatgggaagaatatttcaatccgttcgcaaaagccaaagaaatagctagtcagatactagctgatagaaagaaggcgttggttctgtctattcaaggacaatctgaattgccagaatcaatgcggctgatttatcttgaaaaactaaataatctctataatcaagggattctatctattcaaaagacagaaagttctgagatgctaagtggtgcattggaaaatggtttaaatagtttaaagagtttagattttcctatttcagaagttggaaatgctttggcaccagatttatcagtaggtgatcgctcaacggtttcagatgttgattctctatcatctcaagaaacaagttccacaaatttggaagcagacacagagaatgcaggtattattgcagatggtaccaatcaattgcattttccagtggaggcccaaacgacatcttcagtagaggctgagggagataatgtttttgaacaagaggcagatacattaccaataattattgaaaacaaggatgaatttggttcagaactatcaggaaacatgcaaacgtcagaaacggattcgctagtagtagctgttgaagaagatgtgaaaaatgatgaggtagaccaagttgaaaagcttcttgaatcagaaaaagttgaaaatcagagttcggaacttctgtcagacaccctaatcgtagagggtgcaaatgacaaagaagaagatagagtggaggcggttgtttctgaacaaccagactcaataccacatcaaaatgtagaaatctctcctgtagaaccaatgaatgtcgaaactgaatctgtggtcactcctattaatgatgcagctactcctcatggtttcccgatgtatatagataattccgtaactgaatctgtagctactccacttgaaaaagactccattcaagccggagagacagaaattgcagaaccaacctcgagcgaatcaactagtgttgaagctgaacttgtcgacaattctgaaatccattcagctacctcttcagttactccccgtggttcctcggcatatgcagatagttccacaactgaatctgtagctactctgcttgaaaaagactccattcaggctggagagacagaaattgcagaaccaacctcgagcaaatcaactaatgtcgaagctgcatctgtcgacaattctgaaattcatgcagatacctctctaactgctgtttcatcagtcaatctggataatccagtgattgaaccagtagctatcccccttatcggttctaagagggacacgaatgcagaagtggaagtttcttcattatcgaaaagagaggttagaaaaccaaatactgaagggctaatctctgttcaatcaaaagttattaagaaagaattgctagaatcaagcttagtagaagcagggtctccattgctagaagccaccattgctcagtcttcaaactcaaatagtactgagataggtatgagctatcagaatactgtgttattagagtctaataatacagagcgtcaggtgtctaaagcagaaattgttatagaacacaaggagacagagttagttgaaacggtttcatctgcttctgagcctgtagtgctcgtagaaaatatctcacaaacctcaaataatactattgaatctggtaagaatatgggagttcaatctcaagcaggtgcaaaacaaattttaggcatagaacaatcttcgaaagtaagtacacctacttcaagacagattatgggagtcggtctattgactcttgttcttggtagtgctttaggtttgttaaagaaaagacgtaagtaa

SEQ ID NO: 10 - protein, 335 aa, synthetic construct
  REGION 1..335: note = amino acids 91 to 425 of WP_044671938
MKVDRGTENVVSRNDTEVTTSEQNQIEVTETKEILNQTSYQTESGEQRQIIWAHGITPPAMEQSGGFVKEKYGDYLNYTAPFKAGKGYYDTNKSLNASFIDLNLCFAAVSSNMVHWWLEQNSSYVERYLKEKKGTVNVGENYAITDLRRYIDSFQDQQNSRVFDMFKTYYGYRTNGFVSDALVDLFINGYKPKVQGGVNLEDSQLVPDSRGGFFYDVFKEKKLTNRIFSGSYERFGEDVRTVLESKGLLGLTYRTLGYATHIVTVWGAEYDNQGKIKAVYITDSDDQQEQIGLKRMGITRDASGNPRLNNHMKNNSAGALLDYVHTIRLGQDLWE

SEQ ID NO: 11 - protein, 335 aa, synthetic construct
  REGION 1..335: note = amino acids 91 to 425 of WP_002935529
MKVDRGTENVVSRNDTEVTTSEQNQIEVTETKEILNQTSYQTESGEQRQIIWAHGITPPAMEQSGGFVKEKYGDYLNYTAPFKAGKGYYDTNKSLNASFIDLNLCFAAVSSNMVHWWLEQNSSYVERYLKEKKGTVNVGENYAITDLRRYIDSFQDQQNSRVFDMFKTYYGYRTNGFVSDALVDLFINGYKPKVQGGVNLEDSQLVPDSRGGFFYDVFKEKKLTNRIFSGSYERFGEDVRTVLESKGLLGLTYRTLGYATHIVTVWGAEYDNQGKIRAVYITDSDDQQEQIGLKRMGITRDASGNPRLNNHVKNNSAGALLDYVHTIRLGQDLWE

SEQ ID NO: 12 - protein, 335 aa, synthetic construct
  REGION 1..335: note = amino acids 92 to 426 of WP_015647040
MKVDRGTENVVSRNDKEVTTSEKNQIEVTETKEILNQTSYQTESGEQRQIIWAHGITPPAMEQSGGFVKEKYGDYLNYTAPFEAGKGYYDTNKSLNASFIDLNLCFAAVSSNMVHWWLEQNSSYVERYLKEKNSTVNVGENYAITDLRRYINSFQNQQNSRVFDMFKTYYGYRTNGFVSDALVDLFINGYKPKAQGGVNLEDSQLVPDSRGGFFYDVFKEKKLTNRIFSGSYERFGEDVRTVLESKGLLGLTYRTLGYATHIVTVWGAEYDNQGKIKAVYITDSDDQQEQIGLKRMGITRDASGNPRLNNHVKNNSAGALLDYVHTIRLGQDLWE

SEQ ID NO: 13 - protein, 335 aa, synthetic construct
  REGION 1..335: note = amino acids 92 to 426 of WP_023370787
MKSDNGDENAVSRDDSEVTTNEQNQIEVTETKEILNQTSYQTESGEQRQIIWAHGITPPAMEQSGGFVKEKYGDYLNYTAPFEAGKGYYDTNKSLNASFIDLNLCFAAVSSNMVHWWLEQNSSYVERYLKEKKGTVNVEENYAITDIRRYINSFQNQQNSRVFDMFKTYYGYRTNGFVSDALVDLFINGYKPKSQGGVNLEDSHLVPDSRGGFFYDVFKEKKLTNRIFSGSYERFGEDVRTVLESKGLLGLTYRTLGYATHIVTVWGAEYDNQGKIKAVYITDSDDQQEQIGLKRMGITRDASGNPRLNNHMKNNSAGALLDYVHTIRLGQDLWE

SEQ ID NO: 14 - protein, 335 aa, synthetic construct
  REGION 1..335: note = amino acids 92 to 426 of WP_044678723
MNSDNGDENVVSRDDSEVTTNEQNQIEVTETKEILNYTSYQTESGEQRQIVWAYGITPPVMEQKGGFVKEKYGDYLNYTAPFEAGKGYYDTNKSLNASFIDLNLCFAAVSSNMVHWWLEQNSSYVERYLKEKKGTVNVEENYAITDLRRYINSFQNQQNSRVFDMFKTYYGYRTNGFVSDALVDLFINGYKPKAQGGVNLEDSQLVPDSRGGFFYDVFKEKKLTNRIFSGSYERFGEDVRTVLESKGLLGLTYRTLGYATHIVTVWGAEYDNQGKIKAVYITDSDDQQEQIGLKRMGITRDASGNPRLNNHMKNNSAGALLDYVHTIRLGQDLWE